European Patent Application EP 4 151 229 A1, published March 22, 2023. Title: RECOMBINANT FUSION PROTEINS TARGETING CD47 AND PD-L1, PREPARATION AND USE THEREOF. Applicant: ImmuneOnco Biopharmaceuticals (Shanghai) Co., Ltd. The sequence listing filed with the application follows.

SEQUENCE LISTING (23 sequences)

SEQ ID NO: 1 - DNA, 375 bp, Artificial Sequence
  SIRPαD1 mutant
gaggaggagctgcaggtgattcagcctgacaagtccgtatcagttgcagctggagagtcggccattctgcactgcactgtgacctccctgatccctgtggggcccatccagtggttcagaggagctggaccagcccgggaattaatctacaatcaaaaagaaggccacttcccccgggtaacaactgtttcagagtccacaaagagagaaaacatggacttttccatcagcatcagtgccatcaccccagcagatgccggcacctactactgtgtgaagttccggaaagggagccctgacacggagtttaagtctggagcaggcactgagctgtctgtgcgtgccaaaccctctgcccccgtggtatcgggccct

SEQ ID NO: 2 - protein, 125 aa, Artificial Sequence
  SIRPαD1 mutant
EEELQVIQPDKSVSVAAGESAILHCTVTSLIPVGPIQWFRGAGPARELIYNQKEGHFPRVTTVSESTKRENMDFSISISAITPADAGTYYCVKFRKGSPDTEFKSGAGTELSVRAKPSAPVVSGP

SEQ ID NO: 3 - DNA, 45 bp, Artificial Sequence
  Linker
ggcggcggtgggagcggcggcggtgggagcggcggcgggggctcg

SEQ ID NO: 4 - protein, 15 aa, Artificial Sequence
  Linker
GGGGSGGGGSGGGGS

SEQ ID NO: 5 - DNA, 1356 bp, Artificial Sequence
  Heavy chain of anti-PD-L1 antibody IMM2515
caagtgcagctggtgcagagcggcgccgaggtgaagaagcctggcgcaagcgtgaaggtgagctgcaaggcaagcggctacaccttcacaagcaactggatgcactgggtgagacaagcccctggccaaggcctggagtggatgggcatgatccaccctaacagcggcagcagcaactacaacgagaagttcaagagcagagtgaccatgacaagagacacaagcacaagcaccgtgtacatggagctgagcagcctgagaagcgaggacaccgccgtgtactactgcgctagaagctactacggcagcagcccttactacttcgactactggggccaaggcaccctggtgaccgtgagcagcgctagcaccaagggcccatcggtcttccccctggcaccctcctccaagagcacctctgggggcacagcggccctgggctgcctggtcaaggactacttccccgaaccggtgacggtgtcgtggaactcaggcgccctgaccagcggcgtgcacaccttcccggctgtcctacagtcctcaggactctactccctcagcagcgtggtgaccgtgccctccagcagcttgggcacccagacctacatctgcaacgtgaatcacaagcccagcaacaccaaggtggacaagagagttgagcccaaatcttgtgacaaaactcacacatgcccaccgtgcccagcacctgaactcctggggggaccgtcagtcttcctcttccccccaaaacccaaggacaccctcatgatctcccggacccctgaggtcacatgcgtggtggtggacgtgagccacgaagaccctgaggtcaagttcaactggtatgtggacggcgtggaggtgcataatgccaagacaaagccgcgggaggagcagtacaacgccacgtaccgtgtggtcagcgtcctcaccgtcctgcaccaagactggctgaatggcaaggagtacaagtgcaaggtctccaacaaagccctcccagcccccatcgccgcaaccatctccaaagccaaagggcagccccgagaaccacaggtgtacaccctgcccccatcccgggaggagatgaccaagaaccaagtcagcctgacctgcctggtcaaaggcttctatcccagcgacatcgccgtggagtgggagagcaatgggcagccggagaacaactacaagaccacgcctcccgtgctggactccgacggctccttcttcctctattccaagctcaccgtggacaagagcaggtggcagcaggggaacgtcttctcatgctccgtgatgcatgaggctctgcacaaccactacacgcagaagagcctctccctgtctccgggcaaatga

SEQ ID NO: 6 - protein, 451 aa, Artificial Sequence
  Heavy chain of anti-PD-L1 antibody IMM2515
QVQLVQSGAEVKKPGASVKVSCKASGYTFTSNWMHWVRQAPGQGLEWMGMIHPNSGSSNYNEKFKSRVTMTRDTSTSTVYMELSSLRSEDTAVYYCARSYYGSSPYYFDYWGQGTLVTVSSASTKGPSVFPLAPSSKSTSGGTAALGCLVKDYFPEPVTVSWNSGALTSGVHTFPAVLQSSGLYSLSSVVTVPSSSLGTQTYICNVNHKPSNTKVDKRVEPKSCDKTHTCPPCPAPELLGGPSVFLFPPKPKDTLMISRTPEVTCVVVDVSHEDPEVKFNWYVDGVEVHNAKTKPREEQYNATYRVVSVLTVLHQDWLNGKEYKCKVSNKALPAPIAATISKAKGQPREPQVYTLPPSREEMTKNQVSLTCLVKGFYPSDIAVEWESNGQPENNYKTTPPVLDSDGSFFLYSKLTVDKSRWQQGNVFSCSVMHEALHNHYTQKSLSLSPGK

SEQ ID NO: 7 - DNA, 645 bp, Artificial Sequence
  Light chain of anti-PD-L1 antibody IMM2515
gacattcagatgacacagagccctagcagcctgagcgcaagcgtgggcgacagagtgaccatcacctgcagagcaagccaagacatcatcaactacctgaactggtatcagcagaagcctggcaaggcccctaagctgctgatctactacacaagcagactgcacagcggcgtgcctagcagattcagcggcagcggcagcggcaccgacttcaccttcaccatcagcagcctgcagcctgaggacatcgccacctactactgtcagcaaggcgacaccctgccttggaccttcggccaaggcaccaaggtggagatcaagcgaactgtggctgcaccatctgtcttcatcttcccgccatctgatgagcagttgaaatctggaactgcctctgttgtgtgcctgctgaataacttctatcccagagaggccaaagtacagtggaaggtggataacgccctccaatcgggtaactcccaggagagtgtcacagagcaggacagcaaggacagcacctacagcctcagcagcaccctgacgctgagcaaagcagactacgagaaacacaaagtctacgcctgcgaagtcacccatcagggcctgagctcgcccgtcacaaagagcttcaacaggggagagtgttag

SEQ ID NO: 8 - protein, 214 aa, Artificial Sequence
  Light chain of anti-PD-L1 antibody IMM2515
DIQMTQSPSSLSASVGDRVTITCRASQDIINYLNWYQQKPGKAPKLLIYYTSRLHSGVPSRFSGSGSGTDFTFTISSLQPEDIATYYCQQGDTLPWTFGQGTKVEIKRTVAAPSVFIFPPSDEQLKSGTASVVCLLNNFYPREAKVQWKVDNALQSGNSQESVTEQDSKDSTYSLSSTLTLSKADYEKHKVYACEVTHQGLSSPVTKSFNRGEC

SEQ ID NO: 9 - DNA, 1776 bp, Artificial Sequence
  SIRPαD1 mutant-linker-anti-PD-L1 heavy chain
gaggaggagctgcaggtgattcagcctgacaagtccgtatcagttgcagctggagagtcggccattctgcactgcactgtgacctccctgatccctgtggggcccatccagtggttcagaggagctggaccagcccgggaattaatctacaatcaaaaagaaggccacttcccccgggtaacaactgtttcagagtccacaaagagagaaaacatggacttttccatcagcatcagtgccatcaccccagcagatgccggcacctactactgtgtgaagttccggaaagggagccctgacacggagtttaagtctggagcaggcactgagctgtctgtgcgtgccaaaccctctgcccccgtggtatcgggccctggcggcggtgggagcggcggcggtgggagcggcggcgggggctcgcaagtgcagctggtgcagagcggcgccgaggtgaagaagcctggcgcaagcgtgaaggtgagctgcaaggcaagcggctacaccttcacaagcaactggatgcactgggtgagacaagcccctggccaaggcctggagtggatgggcatgatccaccctaacagcggcagcagcaactacaacgagaagttcaagagcagagtgaccatgacaagagacacaagcacaagcaccgtgtacatggagctgagcagcctgagaagcgaggacaccgccgtgtactactgcgctagaagctactacggcagcagcccttactacttcgactactggggccaaggcaccctggtgaccgtgagcagcgctagcaccaagggcccatcggtcttccccctggcaccctcctccaagagcacctctgggggcacagcggccctgggctgcctggtcaaggactacttccccgaaccggtgacggtgtcgtggaactcaggcgccctgaccagcggcgtgcacaccttcccggctgtcctacagtcctcaggactctactccctcagcagcgtggtgaccgtgccctccagcagcttgggcacccagacctacatctgcaacgtgaatcacaagcccagcaacaccaaggtggacaagagagttgagcccaaatcttgtgacaaaactcacacatgcccaccgtgcccagcacctgaactcctggggggaccgtcagtcttcctcttccccccaaaacccaaggacaccctcatgatctcccggacccctgaggtcacatgcgtggtggtggacgtgagccacgaagaccctgaggtcaagttcaactggtatgtggacggcgtggaggtgcataatgccaagacaaagccgcgggaggagcagtacaacgccacgtaccgtgtggtcagcgtcctcaccgtcctgcaccaagactggctgaatggcaaggagtacaagtgcaaggtctccaacaaagccctcccagcccccatcgccgcaaccatctccaaagccaaagggcagccccgagaaccacaggtgtacaccctgcccccatcccgggaggagatgaccaagaaccaagtcagcctgacctgcctggtcaaaggcttctatcccagcgacatcgccgtggagtgggagagcaatgggcagccggagaacaactacaagaccacgcctcccgtgctggactccgacggctccttcttcctctattccaagctcaccgtggacaagagcaggtggcagcaggggaacgtcttctcatgctccgtgatgcatgaggctctgcacaaccactacacgcagaagagcctctccctgtctccgggcaaatga

SEQ ID NO: 10 - protein, 591 aa, Artificial Sequence
  SIRPαD1 mutant-linker-anti-PD-L1 heavy chain
EEELQVIQPDKSVSVAAGESAILHCTVTSLIPVGPIQWFRGAGPARELIYNQKEGHFPRVTTVSESTKRENMDFSISISAITPADAGTYYCVKFRKGSPDTEFKSGAGTELSVRAKPSAPVVSGPGGGGSGGGGSGGGGSQVQLVQSGAEVKKPGASVKVSCKASGYTFTSNWMHWVRQAPGQGLEWMGMIHPNSGSSNYNEKFKSRVTMTRDTSTSTVYMELSSLRSEDTAVYYCARSYYGSSPYYFDYWGQGTLVTVSSASTKGPSVFPLAPSSKSTSGGTAALGCLVKDYFPEPVTVSWNSGALTSGVHTFPAVLQSSGLYSLSSVVTVPSSSLGTQTYICNVNHKPSNTKVDKRVEPKSCDKTHTCPPCPAPELLGGPSVFLFPPKPKDTLMISRTPEVTCVVVDVSHEDPEVKFNWYVDGVEVHNAKTKPREEQYNATYRVVSVLTVLHQDWLNGKEYKCKVSNKALPAPIAATISKAKGQPREPQVYTLPPSREEMTKNQVSLTCLVKGFYPSDIAVEWESNGQPENNYKTTPPVLDSDGSFFLYSKLTVDKSRWQQGNVFSCSVMHEALHNHYTQKSLSLSPGK

SEQ ID NO: 11 - DNA, 1095 bp, Artificial Sequence
  SIRPαD1 mutant-Fc (IMM01)
gaggaggagctgcaggtgattcagcctgacaagtccgtatcagttgcagctggagagtcggccattctgcactgcactgtgacctccctgatccctgtggggcccatccagtggttcagaggagctggaccagcccgggaattaatctacaatcaaaaagaaggccacttcccccgggtaacaactgtttcagagtccacaaagagagaaaacatggacttttccatcagcatcagtgccatcaccccagcagatgccggcacctactactgtgtgaagttccggaaagggagccctgacacggagtttaagtctggagcaggcactgagctgtctgtgcgtgccaaaccctctgcccccgtggtatcgggccctgcggcgagggccacacctcagcacgagcccaaatcttgtgacaaaactcacacatgcccaccgtgcccagcacctgaactcctggggggaccgtcagtcttcctcttccccccaaaacccaaggacaccctcatgatctcccggacccctgaggtcacatgcgtggtggtggacgtgagccacgaagaccctgaggtcaagttcaactggtacgtggacggcgtggaggtgcataatgccaagacaaagccgcgggaggagcagtacaacagcacgtaccgtgtggtcagcgtcctcaccgtcctgcaccaggactggctgaatggcaaggagtacaagtgcaaggtctccaacaaagccctcccagcccccatcgagaaaaccatctccaaagccaaagggcagccccgagaaccacaggtgtacaccctgcccccatcccgggatgagctgaccaagaaccaggtcagcctgacctgcctggtcaaaggcttctatcccagcgacatcgccgtggagtgggagagcaatgggcagccggagaacaactacaagaccacgcctcccgtgctggactccgacggctccttcttcctctacagcaagctcaccgtggacaagagcaggtggcagcaggggaacgtcttctcatgctccgtgatgcatgaggctctgcacaaccactacacgcagaagagcctctccctgtctccgggttga

SEQ ID NO: 12 - protein, 364 aa, Artificial Sequence
  SIRPαD1 mutant-Fc (IMM01)
EEELQVIQPDKSVSVAAGESAILHCTVTSLIPVGPIQWFRGAGPARELIYNQKEGHFPRVTTVSESTKRENMDFSISISAITPADAGTYYCVKFRKGSPDTEFKSGAGTELSVRAKPSAPVVSGPAARATPQHEPKSCDKTHTCPPCPAPELLGGPSVFLFPPKPKDTLMISRTPEVTCVVVDVSHEDPEVKFNWYVDGVEVHNAKTKPREEQYNSTYRVVSVLTVLHQDWLNGKEYKCKVSNKALPAPIEKTISKAKGQPREPQVYTLPPSRDELTKNQVSLTCLVKGFYPSDIAVEWESNGQPENNYKTTPPVLDSDGSFFLYSKLTVDKSRWQQGNVFSCSVMHEALHNHYTQKSLSLSPG

SEQ ID NO: 13 - DNA, 57 bp, Mus musculus
atgggatggtcatgtatcatcctttttctggtagcaactgcaactggagtacattca

SEQ ID NO: 14 - DNA, 9 bp, Artificial Sequence
  Kozak
gccgccacc

SEQ ID NO: 15 - DNA, 1204 bp, Artificial Sequence
  SIRPαD1 mutant-linker-anti-PD-L1 light chain
gaggaggagctgcaggtgattcagcctgacaagtccgtatcagttgcagctggagagtcggccattctgcactgcactgtgacctccctgatccctgtggggcccatccagtggttcagaggagctggaccagcccgggaattaatctacaatcaaaaagaaggccacttcccccgggtaacaactgtttcagagtccacaaagagagaaaacatggacttttccatcagcatcagtgccatcaccccagcagatgccggcacctactactgtgtgaagttccggaaagggagccctgacacggagtttaagtctggagcaggcactgagctgtctgtgcgtgccaaaccctctgcccccgtggtatcgggccctggcggcggtgggagcggcggcggtgggagcggcggcgggggctcggacattcagatgacacagagccctagcagcctgagcgcaagcgtgggcgacagagtgaccatcacctgcagagcaagccaagacatcatcaactacctgaactggtatcagcagaagcctggcaaggcccctaagctgctgatctactacacaagcagactgcacagcggcgtgcctagcagattcagcggcagcggcagcggcaccgacttcaccttcaccatcagcagcctgcagcctgaggacatcgccacctactactgtcagcaaggcgacaccctgccttggaccttcggccaaggcaccaaggtggagatcaagcgtgagttctagaggatccatctgggataagcatgctgttttctgtctgtccctaacatgccctgtgattatccgcaaacaacacacccaagggcagaactttgttacttaaacaccatcctgtttgcttctttcctcaggaactgtggctgcaccatctgtcttcatcttcccgccatctgatgagcagttgaaatctggaactgcctctgttgtgtgcctgctgaataacttctatcccagagaggccaaagtacagtggaaggtggataacgccctccaatcgggtaactcccaggagagtgtcacagagcaggacagcaaggacagcacctacagcctcagcagcaccctgacgctgagcaaagcagactacgagaaacacaaagtctacgcctgcgaagtcacccatcagggcctgagctcgcccgtcacaaagagcttcaacaggggagagtgttag

SEQ ID NO: 16 - protein, 354 aa, Artificial Sequence
  SIRPαD1 mutant-linker-anti-PD-L1 light chain
EEELQVIQPDKSVSVAAGESAILHCTVTSLIPVGPIQWFRGAGPARELIYNQKEGHFPRVTTVSESTKRENMDFSISISAITPADAGTYYCVKFRKGSPDTEFKSGAGTELSVRAKPSAPVVSGPGGGGSGGGGSGGGGSDIQMTQSPSSLSASVGDRVTITCRASQDIINYLNWYQQKPGKAPKLLIYYTSRLHSGVPSRFSGSGSGTDFTFTISSLQPEDIATYYCQQGDTLPWTFGQGTKVEIKRTVAAPSVFIFPPSDEQLKSGTASVVCLLNNFYPREAKVQWKVDNALQSGNSQESVTEQDSKDSTYSLSSTLTLSKADYEKHKVYACEVTHQGLSSPVTKSFNRGEC

SEQ ID NO: 17 - protein, 10 aa, Artificial Sequence
  Linker
GGGGSGGGGS

SEQ ID NO: 18 - protein, 20 aa, Artificial Sequence
  Linker
GGGGSGGGGSGGGGSGGGGS

SEQ ID NO: 19 - protein, 121 aa, Artificial Sequence
  Heavy chain variable region of anti-PD-L1 antibody IMM2515
QVQLVQSGAEVKKPGASVKVSCKASGYTFTSNWMHWVRQAPGQGLEWMGMIHPNSGSSNYNEKFKSRVTMTRDTSTSTVYMELSSLRSEDTAVYYCARSYYGSSPYYFDYWGQGTLVTVSS

SEQ ID NO: 20 - protein, 107 aa, Artificial Sequence
  Light chain variable region of anti-PD-L1 antibody IMM2515
DIQMTQSPSSLSASVGDRVTITCRASQDIINYLNWYQQKPGKAPKLLIYYTSRLHSGVPSRFSGSGSGTDFTFTISSLQPEDIATYYCQQGDTLPWTFGQGTKVEIK

SEQ ID NO: 21 - protein, 330 aa, Artificial Sequence
  Heavy chain constant region
ASTKGPSVFPLAPSSKSTSGGTAALGCLVKDYFPEPVTVSWNSGALTSGVHTFPAVLQSSGLYSLSSVVTVPSSSLGTQTYICNVNHKPSNTKVDKRVEPKSCDKTHTCPPCPAPELLGGPSVFLFPPKPKDTLMISRTPEVTCVVVDVSHEDPEVKFNWYVDGVEVHNAKTKPREEQYNATYRVVSVLTVLHQDWLNGKEYKCKVSNKALPAPIAATISKAKGQPREPQVYTLPPSREEMTKNQVSLTCLVKGFYPSDIAVEWESNGQPENNYKTTPPVLDSDGSFFLYSKLTVDKSRWQQGNVFSCSVMHEALHNHYTQKSLSLSPGK

SEQ ID NO: 22 - protein, 391 aa, Artificial Sequence
  Human PD-1-mouse IgG1 Fc
MGWSCIILFLVATATGVHSLDSPDRPWNPPTFSPALLVVTEGDAATFTCSFSNTSESFVLNWYRMSPSNQTDKLAAFPEDRSQPGQDCRFRVTQLPNGRDFHMSVVRARRNDSGTYLCGAISLAPKAQIKESLRAELRVTERRAEVPTAHPSPSPRPAGQFQEFVPRDCGCKPCICTVPEVSSVFIFPPKPKDVLTITLTPKVTCVVVDISKDDPEVQFSWFVDDVEVHTAQTQPREEQFNSTFRSVSELPIMHQDWLNGKEFKCRVNSAAFPAPIEKTISKTKGRPKAPQVYTIPPPKEQMAKDKVSLTCMITDFFPEDITVEWQWNGQPAENYKNTQPIMNTNGSYFVYSKLNVQKSNWEAGNTFTCSVLHEGLHNHHTEKSLSHSPGK

SEQ ID NO: 23 - protein, 602 aa, Artificial Sequence
  Wild type human SIRPαD1-human IgG1 Fc
MGWSCIILFLVATATGVHSSCAWSGVAGEEELQVIQPDKSVSVAAGESAILHCTVTSLIPVGPIQWFRGAGPARELIYNQKEGHFPRVTTVSESTKRENMDFSISISNITPADAGTYYCVKFRKGSPDTEFKSGAGTELSVRAKPSAPVVSGPAARATPQHTVSFTCESHGFSPRDITLKWFKNGNELSDFQTNVDPVGESVSYSIHSTAKVVLTREDVHSQVICEVAHVTLQGDPLRGTANLSETIRVPPTLEVTQQPVRAENQVNVTCQVRKFYPQRLQLTWLENGNVSRTETASTVTENKDGTYNWMSWLLVNVSAHRDDVKLTCQVEHDGQPAVSKSHDLKVSAHPKEQGSNTAAENTGSNERNEFEPKSCDKTHTCPPCPAPELLGGPSVFLFPPKPKDTLMISRTPEVTCVVVDVSHEDPEVKFNWYVDGVEVHNAKTKPREEQYNSTYRVVSVLTVLHQDWLNGKEYKCKVSNKALPAPIEKTISKAKGQPREPQVYTLPPSRDELTKNQVSLTCLVKGFYPSDIAVEWESNGQPENNYKTTPPVLDSDGSFFLYSKLTVDKSRWQQGNVFSCSVMHEALHNHYTQKSLSLSPGK